European Patent Application EP 4 180 522 A9, published July 19, 2023. Title: 一种用于在昆虫细胞中表达包含重叠开放阅读框的基因的表达盒及其应用. Applicant: 武汉枢密脑科学技术有限公司. The sequence listing filed with the application follows.

SEQUENCE LISTING (39 sequences)

SEQ ID NO: 1 - DNA, 110 bp, AcMNPV
  Promoter p10
gacctttaattcaacccaacacaatatattatagttaaataagaattattatcaaatcatttgtatattaattaaaatactatactgtaaattacattttatttacaatc

SEQ ID NO: 2 - DNA, 137 bp, Artificial Sequence
  Intron
gtaagtattcattgtaaatctgatattatttgtattattatacctacctaatttgcagtgcagataaatatgccggatttatcgtgttcgccattagggcagtatattctcattcttccttttcctttttttttcag

SEQ ID NO: 3 - DNA, 108 bp, Artificial Sequence
  Intron
gtaagtatcgataactttgttttctttcacatttacaactccgacatacaaattcaggtatggcccattacggcagtataaattcgttcattttggatattgtttcag

SEQ ID NO: 4 - DNA, 110 bp, Artificial Sequence
  Intron
gtatcgataactttgttttctttcacatctacaacgccgacgccgccatggccatcgtgttcgccattagggcagtatattctcattcttccttttcctttttttttcag

SEQ ID NO: 5 - DNA, 179 bp, Artificial Sequence
  Intron
gtaagtattcattgtaaatctgatattatttgtattattatacctacctaatttgcagtgcagataaatatgccggatggtaattttattactgtttggtccataaacacttgtttaccatttccttttttacaagttttaatatgttctgcatatataaaacattatgtattttgcag

SEQ ID NO: 6 - DNA, 54 bp, Thosea asigna virus
  Self-cleaving peptides T2A
gaagggcggggaagcctcctaacctgcggtgacgttgaggaaaatccgggtcca

SEQ ID NO: 7 - DNA, 2211 bp, Artificial Sequence
  Cap ORF
atggctgccgacggttatctacccgattggctcgaggacaaccttagtgaaggaattcgcgagtggtgggctttgaaacctggagcccctcaacccaaggcaaatcaacaacatcaagacaacgctcgaggtcttgtgcttccgggttacaaataccttggacccggcaacggactcgacaagggggagccggtcaacgcagcagacgcggcggccctcgagcacgacaaggcctacgaccagcagctcaaggccggagacaacccgtacctcaagtacaaccacgccgacgccgagttccaggagcggctcaaagaagatacgtcttttgggggcaacctcgggcgagcagtcttccaggccaaaaagaggcttcttgaacctcttggtctggttgaggaagcggctaagacggctcctggaaagaagaggcctgtagagcagtctcctcaggaaccggactcctccgcgggtattggcaaatcgggtgcacagcccgctaaaaagagactcaatttcggtcagactggcgacacagagtcagtcccagaccctcaaccaatcggagaacctcccgcagccccctcaggtgtgggatctcttacaatggcttcaggtggtggcgcaccagtggcagacaataacgaaggtgccgatggagtgggtagttcctcgggaaattggcattgcgattcccaatggctgggggacagagtcatcaccaccagcacccgaacctgggccctgcccacctacaacaatcacctctacaagcaaatctccaacagcacatctggaggatcttcaaatgacaacgcctacttcggctacagcaccccctgggggtattttgacttcaacagattccactgccacttctcaccacgtgactggcagcgactcatcaacaacaactggggattccggcctaagcgactcaacttcaagctcttcaacattcaggtcaaagaggttacggacaacaatggagtcaagaccatcgccaataaccttaccagcacggtccaggtcttcacggactcagactatcagctcccgtacgtgctcgggtcggctcacgagggctgcctcccgccgttcccagcggacgttttcatgattcctcagtacgggtatctgacgcttaatgatggaagccaggccgtgggtcgttcgtccttttactgcctggaatatttcccgtcgcaaatgctaagaacgggtaacaacttccagttcagctacgagtttgagaacgtacctttccatagcagctacgctcacagccaaagcctggaccgactaatgaatccactcatcgaccaatacttgtactatctctcaaagactattaacggttctggacagaatcaacaaacgctaaaattcagtgtggccggacccagcaacatggctgtccagggaagaaactacatacctggacccagctaccgacaacaacgtgtctcaaccactgtgactcaaaacaacaacagcgaatttgcttggcctggagcttcttcttgggctctcaatggacgtaatagcttgatgaatcctggacctgctatggccagccacaaagaaggagaggaccgtttctttcctttgtctggatctttaatttttggcaaacaaggaactggaagagacaacgtggatgcggacaaagtcatgataaccaacgaagaagaaattaaaactactaacccggtagcaacggagtcctatggacaagtggccacaaaccaccagagtgcccaagcacaggcgcagaccggctgggttcaaaaccaaggaatacttccgggtatggtttggcaggacagagatgtgtacctgcaaggacccatttgggccaaaattcctcacacggacggcaactttcacccttctccgctgatgggagggtttggaatgaagcacccgcctcctcagatcctcatcaaaaacacacctgtacctgcggatcctccaacggccttcaacaaggacaagctgaactctttcatcacccagtattctactggccaagtcagcgtggagatcgagtgggagctgcagaaggaaaacagcaagcgctggaacccggagatccagtacacttccaactattacaagtctaataatgttgaatttgctgttaatactgaaggtgtatatagtgaaccccgccccattggcaccagatacctgactcgtaatctgtaa

SEQ ID NO: 8 - DNA, 2566 bp, Artificial Sequence
  Cap gene expression cassette
gacctttaattcaacccaacacaatatattatagttaaataagaattattatcaaatcatttgtatattaattaaaatactatactgtaaattacattttatttacaatcactcgacgaagacttgatcacccgggtaggacaaggtaagtattcattgtaaatctgatattatttgtattattatacctacctaatttgcagtgcagataaatatgccggatttatcgtgttcgccattagggcagtatattctcattcttccttttcctttttttttcaggttcaccttcaacggctcgggagaagggcggggaagcctcctaacctgcggtgacgttgaggaaaatccgggtccagctgccgacggttatctacccgattggctcgaggacaaccttagtgaaggaattcgcgagtggtgggctttgaaacctggagcccctcaacccaaggcaaatcaacaacatcaagacaacgctcgaggtcttgtgcttccgggttacaaataccttggacccggcaacggactcgacaagggggagccggtcaacgcagcagacgcggcggccctcgagcacgacaaggcctacgaccagcagctcaaggccggagacaacccgtacctcaagtacaaccacgccgacgccgagttccaggagcggctcaaagaagatacgtcttttgggggcaacctcgggcgagcagtcttccaggccaaaaagaggcttcttgaacctcttggtctggttgaggaagcggctaagacggctcctggaaagaagaggcctgtagagcagtctcctcaggaaccggactcctccgcgggtattggcaaatcgggtgcacagcccgctaaaaagagactcaatttcggtcagactggcgacacagagtcagtcccagaccctcaaccaatcggagaacctcccgcagccccctcaggtgtgggatctcttacaatggcttcaggtggtggcgcaccagtggcagacaataacgaaggtgccgatggagtgggtagttcctcgggaaattggcattgcgattcccaatggctgggggacagagtcatcaccaccagcacccgaacctgggccctgcccacctacaacaatcacctctacaagcaaatctccaacagcacatctggaggatcttcaaatgacaacgcctacttcggctacagcaccccctgggggtattttgacttcaacagattccactgccacttctcaccacgtgactggcagcgactcatcaacaacaactggggattccggcctaagcgactcaacttcaagctcttcaacattcaggtcaaagaggttacggacaacaatggagtcaagaccatcgccaataaccttaccagcacggtccaggtcttcacggactcagactatcagctcccgtacgtgctcgggtcggctcacgagggctgcctcccgccgttcccagcggacgttttcatgattcctcagtacgggtatctgacgcttaatgatggaagccaggccgtgggtcgttcgtccttttactgcctggaatatttcccgtcgcaaatgctaagaacgggtaacaacttccagttcagctacgagtttgagaacgtacctttccatagcagctacgctcacagccaaagcctggaccgactaatgaatccactcatcgaccaatacttgtactatctctcaaagactattaacggttctggacagaatcaacaaacgctaaaattcagtgtggccggacccagcaacatggctgtccagggaagaaactacatacctggacccagctaccgacaacaacgtgtctcaaccactgtgactcaaaacaacaacagcgaatttgcttggcctggagcttcttcttgggctctcaatggacgtaatagcttgatgaatcctggacctgctatggccagccacaaagaaggagaggaccgtttctttcctttgtctggatctttaatttttggcaaacaaggaactggaagagacaacgtggatgcggacaaagtcatgataaccaacgaagaagaaattaaaactactaacccggtagcaacggagtcctatggacaagtggccacaaaccaccagagtgcccaagcacaggcgcagaccggctgggttcaaaaccaaggaatacttccgggtatggtttggcaggacagagatgtgtacctgcaaggacccatttgggccaaaattcctcacacggacggcaactttcacccttctccgctgatgggagggtttggaatgaagcacccgcctcctcagatcctcatcaaaaacacacctgtacctgcggatcctccaacggccttcaacaaggacaagctgaactctttcatcacccagtattctactggccaagtcagcgtggagatcgagtgggagctgcagaaggaaaacagcaagcgctggaacccggagatccagtacacttccaactattacaagtctaataatgttgaatttgctgttaatactgaaggtgtatatagtgaaccccgccccattggcaccagatacctgactcgtaatctgtaa

SEQ ID NO: 9 - DNA, 2529 bp, Artificial Sequence
  Cap gene expression cassette
gacctttaattcaacccaacacaatatattatagttaaataagaattattatcaaatcatttgtatattaattaaaatactatactgtaaattacattttatttacaatcactcgacgaagacttgatcacccgggcagcaggtaagtatcgataactttgttttctttcacatttacaactccgacatacaaattcaggtatggcccattacggcagtataaattcgttcattttggatattgtttcagttgcaagtggctcgggagaagggcggggaagcctcctaacctgcggtgacgttgaggaaaatccgggtccagctgccgacggttatcttcccgattggctcgaggacaaccttagtgaaggaattcgcgagtggtgggctttgaaacctggagcccctcaacccaaggcaaatcaacaacatcaagacaacgctcgaggtcttgtgcttccgggttacaaataccttggacccggcaacggactcgacaagggggagccggtcaacgcagcagacgcggcggccctcgagcacgacaaggcctacgaccagcagctcaaggccggagacaacccgtacctcaagtacaaccacgccgacgccgagttccaggagcggctcaaagaagatacgtcttttgggggcaacctcgggcgagcagtcttccaggccaaaaagaggcttcttgaacctcttggtctggttgaggaagcggctaagacggctcctggaaagaagaggcctgtagagcagtctcctcaggaaccggactcctccgcgggtattggcaaatcgggtgcacagcccgctaaaaagagactcaatttcggtcagactggcgacacagagtcagtcccagaccctcaaccaatcggagaacctcccgcagccccctcaggtgtgggatctcttacaatggcttcaggtggtggcgcaccagtggcagacaataacgaaggtgccgatggagtgggtagttcctcgggaaattggcattgcgattcccaatggctgggggacagagtcatcaccaccagcacccgaacctgggccctgcccacctacaacaatcacctctacaagcaaatctccaacagcacatctggaggatcttcaaatgacaacgcctacttcggctacagcaccccctgggggtattttgacttcaacagattccactgccacttctcaccacgtgactggcagcgactcatcaacaacaactggggattccggcctaagcgactcaacttcaagctcttcaacattcaggtcaaagaggttacggacaacaatggagtcaagaccatcgccaataaccttaccagcacggtccaggtcttcacggactcagactatcagctcccgtacgtgctcgggtcggctcacgagggctgcctcccgccgttcccagcggacgttttcatgattcctcagtacgggtatctgacgcttaatgatggaagccaggccgtgggtcgttcgtccttttactgcctggaatatttcccgtcgcaaatgctaagaacgggtaacaacttccagttcagctacgagtttgagaacgtacctttccatagcagctacgctcacagccaaagcctggaccgactaatgaatccactcatcgaccaatacttgtactatctctcaaagactattaacggttctggacagaatcaacaaacgctaaaattcagtgtggccggacccagcaacatggctgtccagggaagaaactacatacctggacccagctaccgacaacaacgtgtctcaaccactgtgactcaaaacaacaacagcgaatttgcttggcctggagcttcttcttgggctctcaatggacgtaatagcttgatgaatcctggacctgctatggccagccacaaagaaggagaggaccgtttctttcctttgtctggatctttaatttttggcaaacaaggaactggaagagacaacgtggatgcggacaaagtcatgataaccaacgaagaagaaattaaaactactaacccggtagcaacggagtcctatggacaagtggccacaaaccaccagagtgcccaagcacaggcgcagaccggctgggttcaaaaccaaggaatacttccgggtatggtttggcaggacagagatgtgtacctgcaaggacccatttgggccaaaattcctcacacggacggcaactttcacccttctccgctgatgggagggtttggaatgaagcacccgcctcctcagatcctcatcaaaaacacacctgtacctgcggatcctccaacggccttcaacaaggacaagctgaactctttcatcacccagtattctactggccaagtcagcgtggagatcgagtgggagctgcagaaggaaaacagcaagcgctggaacccggagatccagtacacttccaactattacaagtctaataatgttgaatttgctgttaatactgaaggtgtatatagtgaaccccgccccattggcaccagatacctgactcgtaatctgtaa

SEQ ID NO: 10 - DNA, 2527 bp, Artificial Sequence
  Cap gene expression cassette
gacctttaattcaacccaacacaatatattatagttaaataagaattattatcaaatcatttgtatattaattaaaatactatactgtaaattacattttatttacaatcactcgacgaagacttgatcacccgggcaggtaagtatcgataactttgttttctttcacatctacaacgccgacgccgccatggccatcgtgttcgccattagggcagtatattctcattcttccttttcctttttttttcaggttggctcgggagaagggcggggaagcctcctaacctgcggtgacgttgaggaaaatccgggtccagctgccgacggttatctacccgattggctcgaggacaaccttagtgaaggaattcgcgagtggtgggctttgaaacctggagcccctcaacccaaggcaaatcaacaacatcaagacaacgctcgaggtcttgtgcttccgggttacaaataccttggacccggcaacggactcgacaagggggagccggtcaacgcagcagacgcggcggccctcgagcacgacaaggcctacgaccagcagctcaaggccggagacaacccgtacctcaagtacaaccacgccgacgccgagttccaggagcggctcaaagaagatacgtcttttgggggcaacctcgggcgagcagtcttccaggccaaaaagaggcttcttgaacctcttggtctggttgaggaagcggctaagacggctcctggaaagaagaggcctgtagagcagtctcctcaggaaccggactcctccgcgggtattggcaaatcgggtgcacagcccgctaaaaagagactcaatttcggtcagactggcgacacagagtcagtcccagaccctcaaccaatcggagaacctcccgcagccccctcaggtgtgggatctcttacaatggcttcaggtggtggcgcaccagtggcagacaataacgaaggtgccgatggagtgggtagttcctcgggaaattggcattgcgattcccaatggctgggggacagagtcatcaccaccagcacccgaacctgggccctgcccacctacaacaatcacctctacaagcaaatctccaacagcacatctggaggatcttcaaatgacaacgcctacttcggctacagcaccccctgggggtattttgacttcaacagattccactgccacttctcaccacgtgactggcagcgactcatcaacaacaactggggattccggcctaagcgactcaacttcaagctcttcaacattcaggtcaaagaggttacggacaacaatggagtcaagaccatcgccaataaccttaccagcacggtccaggtcttcacggactcagactatcagctcccgtacgtgctcgggtcggctcacgagggctgcctcccgccgttcccagcggacgttttcatgattcctcagtacgggtatctgacgcttaatgatggaagccaggccgtgggtcgttcgtccttttactgcctggaatatttcccgtcgcaaatgctaagaacgggtaacaacttccagttcagctacgagtttgagaacgtacctttccatagcagctacgctcacagccaaagcctggaccgactaatgaatccactcatcgaccaatacttgtactatctctcaaagactattaacggttctggacagaatcaacaaacgctaaaattcagtgtggccggacccagcaacatggctgtccagggaagaaactacatacctggacccagctaccgacaacaacgtgtctcaaccactgtgactcaaaacaacaacagcgaatttgcttggcctggagcttcttcttgggctctcaatggacgtaatagcttgatgaatcctggacctgctatggccagccacaaagaaggagaggaccgtttctttcctttgtctggatctttaatttttggcaaacaaggaactggaagagacaacgtggatgcggacaaagtcatgataaccaacgaagaagaaattaaaactactaacccggtagcaacggagtcctatggacaagtggccacaaaccaccagagtgcccaagcacaggcgcagaccggctgggttcaaaaccaaggaatacttccgggtatggtttggcaggacagagatgtgtacctgcaaggacccatttgggccaaaattcctcacacggacggcaactttcacccttctccgctgatgggagggtttggaatgaagcacccgcctcctcagatcctcatcaaaaacacacctgtacctgcggatcctccaacggccttcaacaaggacaagctgaactctttcatcacccagtattctactggccaagtcagcgtggagatcgagtgggagctgcagaaggaaaacagcaagcgctggaacccggagatccagtacacttccaactattacaagtctaataatgttgaatttgctgttaatactgaaggtgtatatagtgaaccccgccccattggcaccagatacctgactcgtaatctgtaa

SEQ ID NO: 11 - DNA, 2605 bp, Artificial Sequence
  Cap gene expression cassette
gacctttaattcaacccaacacaatatattatagttaaataagaattattatcaaatcatttgtatattaattaaaatactatactgtaaattacattttatttacaatcactcgacgaagacttgatcacccgggtaggacaaggtaagtattcattgtaaatctgatattatttgtattattatacctacctaatttgcagtgcagataaatatgccggatggtaattttattactgtttggtccataaacacttgtttaccatttccttttttacaagttttaatatgttctgcatatataaaacattatgtattttgcagcaccttcaacggctcgggagaagggcggggaagcctcctaacctgcggtgacgttgaggaaaatccgggtccagctgccgacggttatctacccgattggctcgaggacaaccttagtgaaggaattcgcgagtggtgggctttgaaacctggagcccctcaacccaaggcaaatcaacaacatcaagacaacgctcgaggtcttgtgcttccgggttacaaataccttggacccggcaacggactcgacaagggggagccggtcaacgcagcagacgcggcggccctcgagcacgacaaggcctacgaccagcagctcaaggccggagacaacccgtacctcaagtacaaccacgccgacgccgagttccaggagcggctcaaagaagatacgtcttttgggggcaacctcgggcgagcagtcttccaggccaaaaagaggcttcttgaacctcttggtctggttgaggaagcggctaagacggctcctggaaagaagaggcctgtagagcagtctcctcaggaaccggactcctccgcgggtattggcaaatcgggtgcacagcccgctaaaaagagactcaatttcggtcagactggcgacacagagtcagtcccagaccctcaaccaatcggagaacctcccgcagccccctcaggtgtgggatctcttacaatggcttcaggtggtggcgcaccagtggcagacaataacgaaggtgccgatggagtgggtagttcctcgggaaattggcattgcgattcccaatggctgggggacagagtcatcaccaccagcacccgaacctgggccctgcccacctacaacaatcacctctacaagcaaatctccaacagcacatctggaggatcttcaaatgacaacgcctacttcggctacagcaccccctgggggtattttgacttcaacagattccactgccacttctcaccacgtgactggcagcgactcatcaacaacaactggggattccggcctaagcgactcaacttcaagctcttcaacattcaggtcaaagaggttacggacaacaatggagtcaagaccatcgccaataaccttaccagcacggtccaggtcttcacggactcagactatcagctcccgtacgtgctcgggtcggctcacgagggctgcctcccgccgttcccagcggacgttttcatgattcctcagtacgggtatctgacgcttaatgatggaagccaggccgtgggtcgttcgtccttttactgcctggaatatttcccgtcgcaaatgctaagaacgggtaacaacttccagttcagctacgagtttgagaacgtacctttccatagcagctacgctcacagccaaagcctggaccgactaatgaatccactcatcgaccaatacttgtactatctctcaaagactattaacggttctggacagaatcaacaaacgctaaaattcagtgtggccggacccagcaacatggctgtccagggaagaaactacatacctggacccagctaccgacaacaacgtgtctcaaccactgtgactcaaaacaacaacagcgaatttgcttggcctggagcttcttcttgggctctcaatggacgtaatagcttgatgaatcctggacctgctatggccagccacaaagaaggagaggaccgtttctttcctttgtctggatctttaatttttggcaaacaaggaactggaagagacaacgtggatgcggacaaagtcatgataaccaacgaagaagaaattaaaactactaacccggtagcaacggagtcctatggacaagtggccacaaaccaccagagtgcccaagcacaggcgcagaccggctgggttcaaaaccaaggaatacttccgggtatggtttggcaggacagagatgtgtacctgcaaggacccatttgggccaaaattcctcacacggacggcaactttcacccttctccgctgatgggagggtttggaatgaagcacccgcctcctcagatcctcatcaaaaacacacctgtacctgcggatcctccaacggccttcaacaaggacaagctgaactctttcatcacccagtattctactggccaagtcagcgtggagatcgagtgggagctgcagaaggaaaacagcaagcgctggaacccggagatccagtacacttccaactattacaagtctaataatgttgaatttgctgttaatactgaaggtgtatatagtgaaccccgccccattggcaccagatacctgactcgtaatctgtaa

SEQ ID NO: 12 - DNA, 92 bp, AcMNPV
  Promoter polh
atcatggagataattaaaatgataaccatctcgcaaataaataagtattttactgttttcgtaacagttttgtaataaaaaaacctataaat

SEQ ID NO: 13 - DNA, 1863 bp, Artificial Sequence
  Rep ORF
atggggttttacgagattgtgattaaggtccccagcgaccttgacgggcatctgcccggcatttctgacagctttgtgaactgggtggccgagaaggagtgggagttgccgccagattctgacttggatctgaatctgattgagcaggcacccctgaccgtggccgagaagctgcagcgcgactttctgacggagtggcgccgtgtgagtaaggccccggaggcccttttctttgtgcaatttgagaagggagagagctacttccacttacacgtgctcgtggaaaccaccggggtgaaatccttagttttgggacgtttcctgagtcagattcgcgaaaaactgattcagagaatttaccgcgggatcgagccgactttgccaaactggttcgcggtcacaaagaccagaaacggcgccggaggcgggaacaaggtggtggacgagtgctacatccccaattacttgctccccaaaacccagcctgagctccagtgggcgtggactaatttagaacagtatttaagcgcctgtttgaatctcacggagcgtaaacggttggtggcgcagcatctgacgcacgtgtcgcagacgcaggagcagaacaaagagaatcagaatcccaattctgacgcgccggtgatcagatcaaaaacttcagccaggtacatggagctggtcgggtggctcgtggacaaggggattacctcggagaagcagtggatccaggaggaccaggcctcatacatctccttcaatgcggcctccaactcgcggtcccaaatcaaggctgccttggacaatgcgggaaagattatgagcctgactaaaaccgcccccgactacctggtgggccagcagcccgtggaggacatttccagcaatcggatttataaaattttggaactaaacgggtacgatccccaatatgcggcttccgtctttctgggatgggccacgaaaaagttcggcaagaggaacaccatctggctgtttgggcctgcaactaccgggaagaccaacatcgcggaggccatagcccacactgtgcccttctacgggtgcgtaaactggaccaatgagaactttcccttcaacgactgtgtcgacaagatggtgatctggtgggaggaggggaagatgaccgccaaggtcgtggagtcggccaaagccattctcggaggaagcaaggtgcgcgtggaccagaaatgcaagtcctcggcccagatagacccgactcccgtgatcgtcacctccaacaccaacatgtgcgccgtgattgacgggaactcaacgaccttcgaacaccagcagccgttgcaagaccggatgttcaaatttgaactcacccgccgtctggatcatgactttgggaaggtcaccaagcaggaagtcaaagactttttccggtgggcaaaggatcacgtggttgaggtggagcatgaattctacgtcaaaaagggtggagccaagaaaagacccgcccccagtgacgcagatataagtgagcccaaacgggtgcgcgagtcagttgcgcagccatcgacgtcagacgcggaagcttcgatcaactacgcagacaggtaccaaaacaaatgttctcgtcacgtgggcatgaatctgatgctgtttccctgcagacaatgcgagagaatgaatcagaattcaaatatctgcttcactcacggacagaaagactgtttagagtgctttcccgtgtcagaatctcaacccgtttctgtcgtcaaaaaggcgtatcagaaactgtgctacattcatcatatcatgggaaaggtgccagacgcttgcactgcctgcgatctggtcaatgtggatttggatgactgcatctttgaacaataa

SEQ ID NO: 14 - DNA, 2255 bp, Artificial Sequence
  Rep gene expression cassette
atcatggagataattaaaatgataaccatctcgcaaataaataagtattttactgttttcgtaacagttttgtaataaaaaaacctataaatattccggattattcataccgtcccaccatcgggcgcggatcctaggacaaggtaagtatgcattgtaaatgtgatattatgtgtattattatacctacctaatttgcagtgcagataaatatgccggatggtaattttattactgtttggtccataaacacttgtttaccatttccttttttacaagttttaatatgttctgcatatataaaacattatgtattttgcagcaccttcaacggctcgggagaagggcggggaagcctcctaacctgcggtgacgttgaggaaaatccgggtccagggttttacgagattgtgattaaggtccccagcgaccttgacgggcatctgcccggcatttctgacagctttgtgaactgggtggccgagaaggagtgggagttgccgccagattctgacttggatctgaatctgattgagcaggcacccctgaccgtggccgagaagctgcagcgcgactttctgacggagtggcgccgtgtgagtaaggccccggaggcccttttctttgtgcaatttgagaagggagagagctacttccacttacacgtgctcgtggaaaccaccggggtgaaatccttagttttgggacgtttcctgagtcagattcgcgaaaaactgattcagagaatttaccgcgggatcgagccgactttgccaaactggttcgcggtcacaaagaccagaaacggcgccggaggcgggaacaaggtggtggacgagtgctacatccccaattacttgctccccaaaacccagcctgagctccagtgggcgtggactaatttagaacagtatttaagcgcctgtttgaatctcacggagcgtaaacggttggtggcgcagcatctgacgcacgtgtcgcagacgcaggagcagaacaaagagaatcagaatcccaattctgacgcgccggtgatcagatcaaaaacttcagccaggtacatggagctggtcgggtggctcgtggacaaggggattacctcggagaagcagtggatccaggaggaccaggcctcatacatctccttcaatgcggcctccaactcgcggtcccaaatcaaggctgccttggacaatgcgggaaagattatgagcctgactaaaaccgcccccgactacctggtgggccagcagcccgtggaggacatttccagcaatcggatttataaaattttggaactaaacgggtacgatccccaatatgcggcttccgtctttctgggatgggccacgaaaaagttcggcaagaggaacaccatctggctgtttgggcctgcaactaccgggaagaccaacatcgcggaggccatagcccacactgtgcccttctacgggtgcgtaaactggaccaatgagaactttcccttcaacgactgtgtcgacaagatggtgatctggtgggaggaggggaagatgaccgccaaggtcgtggagtcggccaaagccattctcggaggaagcaaggtgcgcgtggaccagaaatgcaagtcctcggcccagatagacccgactcccgtgatcgtcacctccaacaccaacatgtgcgccgtgattgacgggaactcaacgaccttcgaacaccagcagccgttgcaagaccggatgttcaaatttgaactcacccgccgtctggatcatgactttgggaaggtcaccaagcaggaagtcaaagactttttccggtgggcaaaggatcacgtggttgaggtggagcatgaattctacgtcaaaaagggtggagccaagaaaagacccgcccccagtgacgcagatataagtgagcccaaacgggtgcgcgagtcagttgcgcagccatcgacgtcagacgcggaagcttcgatcaactacgcagacaggtaccaaaacaaatgttctcgtcacgtgggcatgaatctgatgctgtttccctgcagacaatgcgagagaatgaatcagaattcaaatatctgcttcactcacggacagaaagactgtttagagtgctttcccgtgtcagaatctcaacccgtttctgtcgtcaaaaaggcgtatcagaaactgtgctacattcatcatatcatgggaaaggtgccagacgcttgcactgcctgcgatctggtcaatgtggatttggatgactgcatctttgaacaataa

SEQ ID NO: 15 - DNA, 226 bp, Artificial Sequence
  Intron
gtaagtatcgataactttgttttctttcacatttacaactccgacatacaaatgccgccatggtaagtattcattgtaaatctgatattatttgtattattatacctacctaatttgcagtgcagggtaattttattactgtttggtccataaacacttgtttaccatttccttttttacaagttttaatattttctgcatatataaaacattatttattttgcag

SEQ ID NO: 16 - DNA, 226 bp, Artificial Sequence
  Intron
gtaagtattcattgtaaatctgatattatttgtattattatacctacctaatttgcagtgcaggccgccatggtaagtatcgataactttgttttctttcacatttacaactccgacatacaaattgtaattttattactgtttggtccataaacacttgtttaccatttccttttttacaagttttaatattttctgcatatataaaacattatttattttgcag

SEQ ID NO: 17 - DNA, 2605 bp, Artificial Sequence; identical to SEQ ID NO: 11
  Cap gene expression cassette

SEQ ID NO: 18 - DNA, 2499 bp, Artificial Sequence
  Cap gene expression cassette
gacctttaattcaacccaacacaatatattatagttaaataagaattattatcaaatcatttgtatattaattaaaatactatactgtaaattacattttatttacaatcactcgacgaagacttgatcacccgggtagctaaaggtatttctttgactctaaaaaccttgacgactgtttcgccttgaacaaactaaatgaaccctttatgcaaacagctgcccgtgggctcgggagaagggcggggaagcctcctaacctgcggtgacgttgaggaaaatccgggtccagctgccgacggttatctacccgattggctcgaggacaaccttagtgaaggaattcgcgagtggtgggctttgaaacctggagcccctcaacccaaggcaaatcaacaacatcaagacaacgctcgaggtcttgtgcttccgggttacaaataccttggacccggcaacggactcgacaagggggagccggtcaacgcagcagacgcggcggccctcgagcacgacaaggcctacgaccagcagctcaaggccggagacaacccgtacctcaagtacaaccacgccgacgccgagttccaggagcggctcaaagaagatacgtcttttgggggcaacctcgggcgagcagtcttccaggccaaaaagaggcttcttgaacctcttggtctggttgaggaagcggctaagacggctcctggaaagaagaggcctgtagagcagtctcctcaggaaccggactcctccgcgggtattggcaaatcgggtgcacagcccgctaaaaagagactcaatttcggtcagactggcgacacagagtcagtcccagaccctcaaccaatcggagaacctcccgcagccccctcaggtgtgggatctcttacaatggcttcaggtggtggcgcaccagtggcagacaataacgaaggtgccgatggagtgggtagttcctcgggaaattggcattgcgattcccaatggctgggggacagagtcatcaccaccagcacccgaacctgggccctgcccacctacaacaatcacctctacaagcaaatctccaacagcacatctggaggatcttcaaatgacaacgcctacttcggctacagcaccccctgggggtattttgacttcaacagattccactgccacttctcaccacgtgactggcagcgactcatcaacaacaactggggattccggcctaagcgactcaacttcaagctcttcaacattcaggtcaaagaggttacggacaacaatggagtcaagaccatcgccaataaccttaccagcacggtccaggtcttcacggactcagactatcagctcccgtacgtgctcgggtcggctcacgagggctgcctcccgccgttcccagcggacgttttcatgattcctcagtacgggtatctgacgcttaatgatggaagccaggccgtgggtcgttcgtccttttactgcctggaatatttcccgtcgcaaatgctaagaacgggtaacaacttccagttcagctacgagtttgagaacgtacctttccatagcagctacgctcacagccaaagcctggaccgactaatgaatccactcatcgaccaatacttgtactatctctcaaagactattaacggttctggacagaatcaacaaacgctaaaattcagtgtggccggacccagcaacatggctgtccagggaagaaactacatacctggacccagctaccgacaacaacgtgtctcaaccactgtgactcaaaacaacaacagcgaatttgcttggcctggagcttcttcttgggctctcaatggacgtaatagcttgatgaatcctggacctgctatggccagccacaaagaaggagaggaccgtttctttcctttgtctggatctttaatttttggcaaacaaggaactggaagagacaacgtggatgcggacaaagtcatgataaccaacgaagaagaaattaaaactactaacccggtagcaacggagtcctatggacaagtggccacaaaccaccagagtgcccaagcacaggcgcagaccggctgggttcaaaaccaaggaatacttccgggtatggtttggcaggacagagatgtgtacctgcaaggacccatttgggccaaaattcctcacacggacggcaactttcacccttctccgctgatgggagggtttggaatgaagcacccgcctcctcagatcctcatcaaaaacacacctgtacctgcggatcctccaacggccttcaacaaggacaagctgaactctttcatcacccagtattctactggccaagtcagcgtggagatcgagtgggagctgcagaaggaaaacagcaagcgctggaacccggagatccagtacacttccaactattacaagtctaataatgttgaatttgctgttaatactgaaggtgtatatagtgaaccccgccccattggcaccagatacctgactcgtaatctgtaa

SEQ ID NO: 19 - DNA, 2224 bp, Artificial Sequence
  Rep gene expression cassette
atcatggagataattaaaatgataaccatctcgcaaataaataagtattttactgttttcgtaacagttttgtaataaaaaaacctataaatattccggattattcataccgtcccaccatcgggcgcggatccggacaaggtaagtattcattgtaaatctgatattatttgtattattatacctacctaatttgcagtgcaggccgccatggtaagtatcgataactttgttttctttcacatttacaactccgacatacaaattgtaattttattactgtttggtccataaacacttgtttaccatttccttttttacaagttttaatattttctgcatatataaaacattatttattttgcaggggttttacgagattgtgattaaggtccccagcgaccttgacgggcatctgcccggcatttctgacagctttgtgaactgggtggccgagaaggagtgggagttgccgccagattctgacttggatctgaatctgattgagcaggcacccctgaccgtggccgagaagctgcagcgcgactttctgacggagtggcgccgtgtgagtaaggccccggaggcccttttctttgtgcaatttgagaagggagagagctacttccacttacacgtgctcgtggaaaccaccggggtgaaatccttagttttgggacgtttcctgagtcagattcgcgaaaaactgattcagagaatttaccgcgggatcgagccgactttgccaaactggttcgcggtcacaaagaccagaaacggcgccggaggcgggaacaaggtggtggacgagtgctacatccccaattacttgctccccaaaacccagcctgagctccagtgggcgtggactaatttagaacagtatttaagcgcctgtttgaatctcacggagcgtaaacggttggtggcgcagcatctgacgcacgtgtcgcagacgcaggagcagaacaaagagaatcagaatcccaattctgacgcgccggtgatcagatcaaaaacttcagccaggtacatggagctggtcgggtggctcgtggacaaggggattacctcggagaagcagtggatccaggaggaccaggcctcatacatctccttcaatgcggcctccaactcgcggtcccaaatcaaggctgccttggacaatgcgggaaagattatgagcctgactaaaaccgcccccgactacctggtgggccagcagcccgtggaggacatttccagcaatcggatttataaaattttggaactaaacgggtacgatccccaatatgcggcttccgtctttctgggatgggccacgaaaaagttcggcaagaggaacaccatctggctgtttgggcctgcaactaccgggaagaccaacatcgcggaggccatagcccacactgtgcccttctacgggtgcgtaaactggaccaatgagaactttcccttcaacgactgtgtcgacaagatggtgatctggtgggaggaggggaagatgaccgccaaggtcgtggagtcggccaaagccattctcggaggaagcaaggtgcgcgtggaccagaaatgcaagtcctcggcccagatagacccgactcccgtgatcgtcacctccaacaccaacatgtgcgccgtgattgacgggaactcaacgaccttcgaacaccagcagccgttgcaagaccggatgttcaaatttgaactcacccgccgtctggatcatgactttgggaaggtcaccaagcaggaagtcaaagactttttccggtgggcaaaggatcacgtggttgaggtggagcatgaattctacgtcaaaaagggtggagccaagaaaagacccgcccccagtgacgcagatataagtgagcccaaacgggtgcgcgagtcagttgcgcagccatcgacgtcagacgcggaagcttcgatcaactacgcagacaggtaccaaaacaaatgttctcgtcacgtgggcatgaatctgatgctgtttccctgcagacaatgcgagagaatgaatcagaattcaaatatctgcttcactcacggacagaaagactgtttagagtgctttcccgtgtcagaatctcaacccgtttctgtcgtcaaaaaggcgtatcagaaactgtgctacattcatcatatcatgggaaaggtgccagacgcttgcactgcctgcgatctggtcaatgtggatttggatgactgcatctttgaacaa

SEQ ID NO: 20 - DNA, 98 bp, Artificial Sequence
  Intron
gtaagtatcgataactttgttttctttcacatttacaactccgacatacaaatcccattacggcagtataaattcgttcattttggatattgtttcag

SEQ ID NO: 21 - DNA, 108 bp, Artificial Sequence
  Intron
gtaagtattcattgtaaatctgatattatttgtattattatacctacctaatttgcagtgcagcccattacggcagtataaattcgttcattttggatattgtttcag

SEQ ID NO: 22 - DNA, 2451 bp, Artificial Sequence
  Cap gene expression cassette
gacctttaattcaacccaacacaatatattatagttaaataagaattattatcaaatcatttgtatattaattaaaatactatactgtaaattacattttatttacaatcactcgacgaagacttgatcacccgggtcaggtagtaagtatcgataactttgttttctttcacatttacaactccgacatacaaatcccattacggcagtataaattcgttcattttggatattgtttcagtggctgccgacggttatctacccgattggctcgaggacaaccttagtgaaggaattcgcgagtggtgggctttgaaacctggagcccctcaacccaaggcaaatcaacaacatcaagacaacgctcgaggtcttgtgcttccgggttacaaataccttggacccggcaacggactcgacaagggggagccggtcaacgcagcagacgcggcggccctcgagcacgacaaggcctacgaccagcagctcaaggccggagacaacccgtacctcaagtacaaccacgccgacgccgagttccaggagcggctcaaagaagatacgtcttttgggggcaacctcgggcgagcagtcttccaggccaaaaagaggcttcttgaacctcttggtctggttgaggaagcggctaagacggctcctggaaagaagaggcctgtagagcagtctcctcaggaaccggactcctccgcgggtattggcaaatcgggtgcacagcccgctaaaaagagactcaatttcggtcagactggcgacacagagtcagtcccagaccctcaaccaatcggagaacctcccgcagccccctcaggtgtgggatctcttacaatggcttcaggtggtggcgcaccagtggcagacaataacgaaggtgccgatggagtgggtagttcctcgggaaattggcattgcgattcccaatggctgggggacagagtcatcaccaccagcacccgaacctgggccctgcccacctacaacaatcacctctacaagcaaatctccaacagcacatctggaggatcttcaaatgacaacgcctacttcggctacagcaccccctgggggtattttgacttcaacagattccactgccacttctcaccacgtgactggcagcgactcatcaacaacaactggggattccggcctaagcgactcaacttcaagctcttcaacattcaggtcaaagaggttacggacaacaatggagtcaagaccatcgccaataaccttaccagcacggtccaggtcttcacggactcagactatcagctcccgtacgtgctcgggtcggctcacgagggctgcctcccgccgttcccagcggacgttttcatgattcctcagtacgggtatctgacgcttaatgatggaagccaggccgtgggtcgttcgtccttttactgcctggaatatttcccgtcgcaaatgctaagaacgggtaacaacttccagttcagctacgagtttgagaacgtacctttccatagcagctacgctcacagccaaagcctggaccgactaatgaatccactcatcgaccaatacttgtactatctctcaaagactattaacggttctggacagaatcaacaaacgctaaaattcagtgtggccggacccagcaacatggctgtccagggaagaaactacatacctggacccagctaccgacaacaacgtgtctcaaccactgtgactcaaaacaacaacagcgaatttgcttggcctggagcttcttcttgggctctcaatggacgtaatagcttgatgaatcctggacctgctatggccagccacaaagaaggagaggaccgtttctttcctttgtctggatctttaatttttggcaaacaaggaactggaagagacaacgtggatgcggacaaagtcatgataaccaacgaagaagaaattaaaactactaacccggtagcaacggagtcctatggacaagtggccacaaaccaccagagtgcccaagcacaggcgcagaccggctgggttcaaaaccaaggaatacttccgggtatggtttggcaggacagagatgtgtacctgcaaggacccatttgggccaaaattcctcacacggacggcaactttcacccttctccgctgatgggagggtttggaatgaagcacccgcctcctcagatcctcatcaaaaacacacctgtacctgcggatcctccaacggccttcaacaaggacaagctgaactctttcatcacccagtattctactggccaagtcagcgtggagatcgagtgggagctgcagaaggaaaacagcaagcgctggaacccggagatccagtacacttccaactattacaagtctaataatgttgaatttgctgttaatactgaaggtgtatatagtgaaccccgccccattggcaccagatacctgactcgtaatctgtaa

SEQ ID NO: 23 - DNA, 2461 bp, Artificial Sequence
  Cap gene expression cassette
gacctttaattcaacccaacacaatatattatagttaaataagaattattatcaaatcatttgtatattaattaaaatactatactgtaaattacattttatttacaatcactcgacgaagacttgatcacccggggccgccagtaagtattcattgtaaatctgatattatttgtattattatacctacctaatttgcagtgcagcccattacggcagtataaattcgttcattttggatattgtttcagtggctgccgacggttatctacccgattggctcgaggacaaccttagtgaaggaattcgcgagtggtgggctttgaaacctggagcccctcaacccaaggcaaatcaacaacatcaagacaacgctcgaggtcttgtgcttccgggttacaaataccttggacccggcaacggactcgacaagggggagccggtcaacgcagcagacgcggcggccctcgagcacgacaaggcctacgaccagcagctcaaggccggagacaacccgtacctcaagtacaaccacgccgacgccgagttccaggagcggctcaaagaagatacgtcttttgggggcaacctcgggcgagcagtcttccaggccaaaaagaggcttcttgaacctcttggtctggttgaggaagcggctaagacggctcctggaaagaagaggcctgtagagcagtctcctcaggaaccggactcctccgcgggtattggcaaatcgggtgcacagcccgctaaaaagagactcaatttcggtcagactggcgacacagagtcagtcccagaccctcaaccaatcggagaacctcccgcagccccctcaggtgtgggatctcttacaatggcttcaggtggtggcgcaccagtggcagacaataacgaaggtgccgatggagtgggtagttcctcgggaaattggcattgcgattcccaatggctgggggacagagtcatcaccaccagcacccgaacctgggccctgcccacctacaacaatcacctctacaagcaaatctccaacagcacatctggaggatcttcaaatgacaacgcctacttcggctacagcaccccctgggggtattttgacttcaacagattccactgccacttctcaccacgtgactggcagcgactcatcaacaacaactggggattccggcctaagcgactcaacttcaagctcttcaacattcaggtcaaagaggttacggacaacaatggagtcaagaccatcgccaataaccttaccagcacggtccaggtcttcacggactcagactatcagctcccgtacgtgctcgggtcggctcacgagggctgcctcccgccgttcccagcggacgttttcatgattcctcagtacgggtatctgacgcttaatgatggaagccaggccgtgggtcgttcgtccttttactgcctggaatatttcccgtcgcaaatgctaagaacgggtaacaacttccagttcagctacgagtttgagaacgtacctttccatagcagctacgctcacagccaaagcctggaccgactaatgaatccactcatcgaccaatacttgtactatctctcaaagactattaacggttctggacagaatcaacaaacgctaaaattcagtgtggccggacccagcaacatggctgtccagggaagaaactacatacctggacccagctaccgacaacaacgtgtctcaaccactgtgactcaaaacaacaacagcgaatttgcttggcctggagcttcttcttgggctctcaatggacgtaatagcttgatgaatcctggacctgctatggccagccacaaagaaggagaggaccgtttctttcctttgtctggatctttaatttttggcaaacaaggaactggaagagacaacgtggatgcggacaaagtcatgataaccaacgaagaagaaattaaaactactaacccggtagcaacggagtcctatggacaagtggccacaaaccaccagagtgcccaagcacaggcgcagaccggctgggttcaaaaccaaggaatacttccgggtatggtttggcaggacagagatgtgtacctgcaaggacccatttgggccaaaattcctcacacggacggcaactttcacccttctccgctgatgggagggtttggaatgaagcacccgcctcctcagatcctcatcaaaaacacacctgtacctgcggatcctccaacggccttcaacaaggacaagctgaactctttcatcacccagtattctactggccaagtcagcgtggagatcgagtgggagctgcagaaggaaaacagcaagcgctggaacccggagatccagtacacttccaactattacaagtctaataatgttgaatttgctgttaatactgaaggtgtatatagtgaaccccgccccattggcaccagatacctgactcgtaatctgtaa

SEQ ID NO: 24 - DNA, 2111 bp, Artificial Sequence
  Rep gene expression cassette
atcatggagataattaaaatgataaccatctcgcaaataaataagtattttactgttttcgtaacagttttgtaataaaaaaacctataaatattccggattattcataccgtcccaccatcgggcgcggatcctcaggtagtaagtattcattgtaaatctgatattatttgtattattatacctacctaatttgcagtgcagcccattacggcagtataaattcgttcattttggatattgtttcagtggggttttacgagattgtgattaaggtccccagcgaccttgacgggcatctgcccggcatttctgacagctttgtgaactgggtggccgagaaggagtgggagttgccgccagattctgacttggatctgaatctgattgagcaggcacccctgaccgtggccgagaagctgcagcgcgactttctgacggagtggcgccgtgtgagtaaggccccggaggcccttttctttgtgcaatttgagaagggagagagctacttccacttacacgtgctcgtggaaaccaccggggtgaaatccttagttttgggacgtttcctgagtcagattcgcgaaaaactgattcagagaatttaccgcgggatcgagccgactttgccaaactggttcgcggtcacaaagaccagaaacggcgccggaggcgggaacaaggtggtggacgagtgctacatccccaattacttgctccccaaaacccagcctgagctccagtgggcgtggactaatttagaacagtatttaagcgcctgtttgaatctcacggagcgtaaacggttggtggcgcagcatctgacgcacgtgtcgcagacgcaggagcagaacaaagagaatcagaatcccaattctgacgcgccggtgatcagatcaaaaacttcagccaggtacatggagctggtcgggtggctcgtggacaaggggattacctcggagaagcagtggatccaggaggaccaggcctcatacatctccttcaatgcggcctccaactcgcggtcccaaatcaaggctgccttggacaatgcgggaaagattatgagcctgactaaaaccgcccccgactacctggtgggccagcagcccgtggaggacatttccagcaatcggatttataaaattttggaactaaacgggtacgatccccaatatgcggcttccgtctttctgggatgggccacgaaaaagttcggcaagaggaacaccatctggctgtttgggcctgcaactaccgggaagaccaacatcgcggaggccatagcccacactgtgcccttctacgggtgcgtaaactggaccaatgagaactttcccttcaacgactgtgtcgacaagatggtgatctggtgggaggaggggaagatgaccgccaaggtcgtggagtcggccaaagccattctcggaggaagcaaggtgcgcgtggaccagaaatgcaagtcctcggcccagatagacccgactcccgtgatcgtcacctccaacaccaacatgtgcgccgtgattgacgggaactcaacgaccttcgaacaccagcagccgttgcaagaccggatgttcaaatttgaactcacccgccgtctggatcatgactttgggaaggtcaccaagcaggaagtcaaagactttttccggtgggcaaaggatcacgtggttgaggtggagcatgaattctacgtcaaaaagggtggagccaagaaaagacccgcccccagtgacgcagatataagtgagcccaaacgggtgcgcgagtcagttgcgcagccatcgacgtcagacgcggaagcttcgatcaactacgcagacaggtaccaaaacaaatgttctcgtcacgtgggcatgaatctgatgctgtttccctgcagacaatgcgagagaatgaatcagaattcaaatatctgcttcactcacggacagaaagactgtttagagtgctttcccgtgtcagaatctcaacccgtttctgtcgtcaaaaaggcgtatcagaaactgtgctacattcatcatatcatgggaaaggtgccagacgcttgcactgcctgcgatctggtcaatgtggatttggatgactgcatctttgaacaataa

SEQ ID NO: 25 - DNA, 2048 bp, Artificial Sequence
  Cap gene expression cassette
atacggacctttaattcaacccaacacaatatattatagttaaataagaattattatcaaatcatttgtatattaattaaaatactatactgtaaattacattttatttacaatcactcgacgaagacttgatcacccggggctaagacggctgccgacggttatctacccgattggctcgaggacaaccttagtgaaggaattcgcgagtggtgggctttgaaacctggagcccctcaacccaaggcaaatcaacaacatcaagacaacgctcgaggtcttgtgcttccgggttacaaataccttggacccggcaacggactcgacaagggggagccggtcaacgcagcagacgcggcggccctcgagcacgacaaggcctacgaccagcagctcaaggccggagacaacccgtacctcaagtacaaccacgccgacgccgagttccaggagcggctcaaagaagatacgtcttttgggggcaacctcgggcgagcagtcttccaggccaaaaagaggcttcttgaacctcttggtctggttgaggaagcggctaagacggctcctggaaagaagaggcctgtagagcagtctcctcaggaaccggactcctccgcgggtattggcaaatcgggtgcacagcccgctaaaaagagactcaatttcggtcagactggcgacacagagtcagtcccagaccctcaaccaatcggagaacctcccgcagccccctcaggtgtgggatctcttacaatggcttcaggtggtggcgcaccagtggcagacaataacgaaggtgccgatggagtgggtagttcctcgggaaattggcattgcgattcccaatggctgggggacagagtcatcaccaccagcacccgaacctgggccctgcccacctacaacaatcacctctacaagcaaatctccaacagcacatctggaggatcttcaaatgacaacgcctacttcggctacagcaccccctgggggtattttgacttcaacagattccactgccacttctcaccacgtgactggcagcgactcatcaacaacaactggggattccggcctaagcgactcaacttcaagctcttcaacattcaggtcaaagaggttacggacaacaatggagtcaagaccatcgccaataaccttaccagcacggtccaggtcttcacggactcagactatcagctcccgtacgtgctcgggtcggctcacgagggctgcctcccgccgttcccagcggacgttttcatgattcctcagtacgggtatctgacgcttaatgatggaagccaggccgtgggtcgttcgtccttttactgcctggaatatttcccgtcgcaaatgctaagaacgggtaacaacttccagttcagctacgagtttgagaacgtacctttccatagcagctacgctcacagccaaagcctggaccgactaatgaatccactcatcgaccaatacttgtactatctctcaaagactattaacggttctggacagaatcaacaaacgctaaaattcagtgtggccggacccagcaacatggctgtccagggaagaaactacatacctggacccagctaccgacaacaacgtgtctcaaccactgtgactcaaaacaacaacagcgaatttgcttggcctggagcttcttcttgggctctcaatggacgtaatagcttgatgaatcctggacctgctatggccagccacaaagaaggagaggaccgtttctttcctttgtctggatctttaatttttggcaaacaaggaactggaagagacaacgtggatgcggacaaagtcatgataaccaacgaagaagaaattaaaactactaacccggtagcaacggagtcctatggacaagtggccacaaaccaccagagtgcccaagcacaggcgcagaccggctgggttcaaaaccaaggaatacttccgggtatggtttggcaggacagagatgtgtacctgcaaggacccatttgggccaaaattcctcacacggacggcaactttcacccttctccgct

SEQ ID NO: 26 - DNA, 4814 bp, Artificial Sequence
  ITR -GOI
cctgcaggcagctgcgcgctcgctcgctcactgaggccgcccgggcaaagcccgggcgtcgggcgacctttggtcgcccggcctcagtgagcgagcgagcgcgcagagagggagtggccaactccatcactaggggttcctgcggccgcacgcgccgcccgtcagtgggcagagcgcacatcgcccacagtccccgagaagttggggggaggggtcggcaattgaaccggtgcctagagaaggtggcgcggggtaaactgggaaagtgatgtcgtgtactggctccgcctttttcccgagggtgggggagaaccgtatataagtgcagtagtcgccgtgaacgttctttttcgcaacgggtttgccgccagaacacgcgtaagggatccgccaccatggtgagcaagggcgaggaggataacatggccatcatcaaggagttcatgcgcttcaaggtgcacatggagggctccgtgaacggccacgagttcgagatcgagggcgagggcgagggccgcccctacgagggcacccagaccgccaagctgaaggtgaccaagggtggccccctgcccttcgcctgggacatcctgtcccctcagttcatgtacggctccaaggcctacgtgaagcaccccgccgacatccccgactacttgaagctgtccttccccgagggcttcaagtgggagcgcgtgatgaacttcgaggacggcggcgtggtgaccgtgacccaggactcctccctgcaggacggcgagttcatctacaaggtgaagctgcgcggcaccaacttcccctccgacggccccgtaatgcagaagaagaccatgggctgggaggcctcctccgagcggatgtaccccgaggacggcgccctgaagggcgagatcaagcagaggctgaagctgaaggacggcggccactacgacgctgaggtcaagaccacctacaaggccaagaagcccgtgcagctgcccggcgcctacaacgtcaacatcaagttggacatcacctcccacaacgaggactacaccatcgtggaacagtacgaacgcgccgagggccgccactccaccggcggcatggacgagctgtacaagtaagaattcgatatcaagcttatcgataatcaacctctggattacaaaatttgtgaaagattgactggtattcttaactatgttgctccttttacgctatgtggatacgctgctttaatgcctttgtatcatgctattgcttcccgtatggctttcattttctcctccttgtataaatcctggttgctgtctctttatgaggagttgtggcccgttgtcaggcaacgtggcgtggtgtgcactgtgtttgctgacgcaacccccactggttggggcattgccaccacctgtcagctcctttccgggactttcgctttccccctccctattgccacggcggaactcatcgccgcctgccttgcccgctgctggacaggggctcggctgttgggcactgacaattccgtggtgttgtcggggaaatcatcgtcctttccttggctgctcgcctgtgttgccacctggattctgcgcgggacgtccttctgctacgtcccttcggccctcaatccagcggaccttccttcccgcggcctgctgccggctctgcggcctcttccgcgtcttcgccttcgccctcagacgagtcggatctccctttgggccgcctccccgcatcgataccgagcgctgctcgagagatctacgggtggcatccctgtgacccctccccagtgcctctcctggccctggaagttgccactccagtgcccaccagccttgtcctaataaaattaagttgcatcattttgtctgactaggtgtccttctataatattatggggtggaggggggtggtatggagcaaggggcaagttgggaagacaacctgtagggcctgcggggtctattgggaaccaagctggagtgcagtggcacaatcttggctcactgcaatctccgcctcctgggttcaagcgattctcctgcctcagcctcccgagttgttgggattccaggcatgcatgaccaggctcagctaatttttgtttttttggtagagacggggtttcaccatattggccaggctggtctccaactcctaatctcaggtgatctacccaccttggcctcccaaattgctgggattacaggcgtgaaccactgctcccttccctgtccttctgattttgtaggtaaccacgtgcggaccgagcggccgcaggaacccctagtgatggagttggccactccctctctgcgcgctcgctcgctcactgaggccgggcgaccaaaggtcgcccgacgcccgggctttgcccgggcggcctcagtgagcgagcgagcgcgcagctgcctgcaggcctgcaggcagctgcgcgctcgctcgctcactgaggccgcccgggcaaagcccgggcgtcgggcgacctttggtcgcccggcctcagtgagcgagcgagcgcgcagagagggagtggccaactccatcactaggggttcctgcggccgcacgcgccgcccgtcagtgggcagagcgcacatcgcccacagtccccgagaagttggggggaggggtcggcaattgaaccggtgcctagagaaggtggcgcggggtaaactgggaaagtgatgtcgtgtactggctccgcctttttcccgagggtgggggagaaccgtatataagtgcagtagtcgccgtgaacgttctttttcgcaacgggtttgccgccagaacacgcgtaagggatccgccaccatggtgagcaagggcgaggaggataacatggccatcatcaaggagttcatgcgcttcaaggtgcacatggagggctccgtgaacggccacgagttcgagatcgagggcgagggcgagggccgcccctacgagggcacccagaccgccaagctgaaggtgaccaagggtggccccctgcccttcgcctgggacatcctgtcccctcagttcatgtacggctccaaggcctacgtgaagcaccccgccgacatccccgactacttgaagctgtccttccccgagggcttcaagtgggagcgcgtgatgaacttcgaggacggcggcgtggtgaccgtgacccaggactcctccctgcaggacggcgagttcatctacaaggtgaagctgcgcggcaccaacttcccctccgacggccccgtaatgcagaagaagaccatgggctgggaggcctcctccgagcggatgtaccccgaggacggcgccctgaagggcgagatcaagcagaggctgaagctgaaggacggcggccactacgacgctgaggtcaagaccacctacaaggccaagaagcccgtgcagctgcccggcgcctacaacgtcaacatcaagttggacatcacctcccacaacgaggactacaccatcgtggaacagtacgaacgcgccgagggccgccactccaccggcggcatggacgagctgtacaagtaagaattcgatatcaagcttatcgataatcaacctctggattacaaaatttgtgaaagattgactggtattcttaactatgttgctccttttacgctatgtggatacgctgctttaatgcctttgtatcatgctattgcttcccgtatggctttcattttctcctccttgtataaatcctggttgctgtctctttatgaggagttgtggcccgttgtcaggcaacgtggcgtggtgtgcactgtgtttgctgacgcaacccccactggttggggcattgccaccacctgtcagctcctttccgggactttcgctttccccctccctattgccacggcggaactcatcgccgcctgccttgcccgctgctggacaggggctcggctgttgggcactgacaattccgtggtgttgtcggggaaatcatcgtcctttccttggctgctcgcctgtgttgccacctggattctgcgcgggacgtccttctgctacgtcccttcggccctcaatccagcggaccttccttcccgcggcctgctgccggctctgcggcctcttccgcgtcttcgccttcgccctcagacgagtcggatctccctttgggccgcctccccgcatcgataccgagcgctgctcgagagatctacgggtggcatccctgtgacccctccccagtgcctctcctggccctggaagttgccactccagtgcccaccagccttgtcctaataaaattaagttgcatcattttgtctgactaggtgtccttctataatattatggggtggaggggggtggtatggagcaaggggcaagttgggaagacaacctgtagggcctgcggggtctattgggaaccaagctggagtgcagtggcacaatcttggctcactgcaatctccgcctcctgggttcaagcgattctcctgcctcagcctcccgagttgttgggattccaggcatgcatgaccaggctcagctaatttttgtttttttggtagagacggggtttcaccatattggccaggctggtctccaactcctaatctcaggtgatctacccaccttggcctcccaaattgctgggattacaggcgtgaaccactgctcccttccctgtccttctgattttgtaggtaaccacgtgcggaccgagcggccgcaggaacccctagtgatggagttggccactccctctctgcgcgctcgctcgctcactgaggccgggcgaccaaaggtcgcccgacgcccgggctttgcccgggcggcctcagtgagcgagcgagcgcgcagctgcctgcagg

SEQ ID NO: 27 - DNA, 2602 bp, Artificial Sequence
  Cap gene expression cassette
gacctttaattcaacccaacacaatatattatagttaaataagaattattatcaaatcatttgtatattaattaaaatactatactgtaaattacattttatttacaatcactcgacgaagacttgatcacccgggtaggacaaggtaagtattcattgtaaatctgatattatttgtattattatacctacctaatttgcagtgcagataaatatgccggatggtaattttattactgtttggtccataaacacttgtttaccatttccttttttacaagttttaatatgttctgcatatataaaacattatgtattttgcagcaccttcaacggctcgggagaagggcggggaagcctcctaacctgcggtgacgttgaggaaaatccgggtccagctgccgacggttatctacccgattggctcgaggacactctctctgaaggaataagacagtggtggaagctcaaacctggcccaccaccaccaaagcccgcagagcggcataaggacgacagcaggggtcttgtgcttcctgggtacaagtacctcggacccttcaacggactcgacaagggagagccggtcaacgaggcagacgccgcggccctcgagcacgacaaagcctacgaccggcagctcgacagcggagacaacccgtacctcaagtacaaccacgccgacgcggagtttcaggagcgccttaaagaagatacgtcttttgggggcaacctcggacgagcagtcttccaggcgaaaaagagggttcttgaacctctgggcctggttgaggaacctgttaagacggctccgggaaaaaagaggccggtagagcactctcctgtggagccagactcctcctcgggaaccggaaaggcgggccagcagcctgcaagaaaaagattgaattttggtcagactggagacgcagactcagtacctgacccccagcctctcggacagccaccagcagccccctctggtctgggaactaatacgatggctacaggcagtggcgcaccaatggcagacaataacgagggcgccgacggagtgggtaattcctcgggaaattggcattgcgattccacatggatgggcgacagagtcatcaccaccagcacccgaacctgggccctgcccacctacaacaaccacctctacaaacaaatttccagccaatcaggagcctcgaacgacaatcactactttggctacagcaccccttgggggtattttgacttcaacagattccactgccacttttcaccacgtgactggcaaagactcatcaacaacaactggggattccgacccaagagactcaacttcaagctctttaacattcaagtcaaagaggtcacgcagaatgacggtacgacgacgattgccaataaccttaccagcacggttcaggtgtttactgactcggagtaccagctcccgtacgtcctcggctcggcgcatcaaggatgcctcccgccgttcccagcagacgtcttcatggtgccacagtatggatacctcaccctgaacaacgggagtcaggcagtaggacgctcttcattttactgcctggagtactttccttctcagatgctgcgtaccggaaacaactttaccttcagctacacttttgaggacgttcctttccacagcagctacgctcacagccagagtctggaccgtctcatgaatcctctcatcgaccagtacctgtattacttgagcagaacaaacactccaagtggaaccaccacgcagtcaaggcttcagttttctcaggccggagcgagtgacattcgggaccagtctaggaactggcttcctggaccctgttaccgccagcagcgagtatcaaagacatctgcggataacaacaacagtgaatactcgtggactggagctaccaagtaccacctcaatggcagagactctctggtgaatccgggcccggccatggcaagccacaaggacgatgaagaaaagttttttcctcagagcggggttctcatctttgggaagcaaggctcagagaaaacaaatgtggacattgaaaaggtcatgattacagacgaagaggaaatcaggacaaccaatcccgtggctacggagcagtatggttctgtatctaccaacctccagagaggcaacagacaagcagctaccgcagatgtcaacacacaaggcgttcttccaggcatggtctggcaggacagagatgtgtaccttcaggggcccatctgggcaaagattccacacacggacggacattttcacccctctcccctcatgggtggattcggacttaaacaccctcctccacagattctcatcaagaacaccccggtacctgcgaatccttcgaccaccttcagtgcggcaaagtttgcttccttcatcacacagtactccacgggacaggtcagcgtggagatcgagtgggagctgcagaaggaaaacagcaaacgctggaatcccgaaattcagtacacttccaactacaacaagtctgttaatgtggactttactgtggacactaatggcgtgtattcagagcctcgccccattggcaccagatacctgactcgtaatctgtaa

SEQ ID NO: 28 - DNA, 2574 bp, Artificial Sequence
  Cap gene expression cassette
gacctttaattcaacccaacacaatatattatagttaaataagaattattatcaaatcatttgtatattaattaaaatactatactgtaaattacattttatttacaatcactcgacgaagacttgatcacccgggggacaaggtaagtattcattgtaaatctgatattatttgtattattatacctacctaatttgcagtgcaggccgccatggtaagtatcgataactttgttttctttcacatttacaactccgacatacaaattgtaattttattactgtttggtccataaacacttgtttaccatttccttttttacaagttttaatattttctgcatatataaaacattatttattttgcaggctgccgacggttatctacccgattggctcgaggacactctctctgaaggaataagacagtggtggaagctcaaacctggcccaccaccaccaaagcccgcagagcggcataaggacgacagcaggggtcttgtgcttcctgggtacaagtacctcggacccttcaacggactcgacaagggagagccggtcaacgaggcagacgccgcggccctcgagcacgacaaagcctacgaccggcagctcgacagcggagacaacccgtacctcaagtacaaccacgccgacgcggagtttcaggagcgccttaaagaagatacgtcttttgggggcaacctcggacgagcagtcttccaggcgaaaaagagggttcttgaacctctgggcctggttgaggaacctgttaagacggctccgggaaaaaagaggccggtagagcactctcctgtggagccagactcctcctcgggaaccggaaaggcgggccagcagcctgcaagaaaaagattgaattttggtcagactggagacgcagactcagtacctgacccccagcctctcggacagccaccagcagccccctctggtctgggaactaatacgatggctacaggcagtggcgcaccaatggcagacaataacgagggcgccgacggagtgggtaattcctcgggaaattggcattgcgattccacatggatgggcgacagagtcatcaccaccagcacccgaacctgggccctgcccacctacaacaaccacctctacaaacaaatttccagccaatcaggagcctcgaacgacaatcactactttggctacagcaccccttgggggtattttgacttcaacagattccactgccacttttcaccacgtgactggcaaagactcatcaacaacaactggggattccgacccaagagactcaacttcaagctctttaacattcaagtcaaagaggtcacgcagaatgacggtacgacgacgattgccaataaccttaccagcacggttcaggtgtttactgactcggagtaccagctcccgtacgtcctcggctcggcgcatcaaggatgcctcccgccgttcccagcagacgtcttcatggtgccacagtatggatacctcaccctgaacaacgggagtcaggcagtaggacgctcttcattttactgcctggagtactttccttctcagatgctgcgtaccggaaacaactttaccttcagctacacttttgaggacgttcctttccacagcagctacgctcacagccagagtctggaccgtctcatgaatcctctcatcgaccagtacctgtattacttgagcagaacaaacactccaagtggaaccaccacgcagtcaaggcttcagttttctcaggccggagcgagtgacattcgggaccagtctaggaactggcttcctggaccctgttaccgccagcagcgagtatcaaagacatctgcggataacaacaacagtgaatactcgtggactggagctaccaagtaccacctcaatggcagagactctctggtgaatccgggcccggccatggcaagccacaaggacgatgaagaaaagttttttcctcagagcggggttctcatctttgggaagcaaggctcagagaaaacaaatgtggacattgaaaaggtcatgattacagacgaagaggaaatcaggacaaccaatcccgtggctacggagcagtatggttctgtatctaccaacctccagagaggcaacagacaagcagctaccgcagatgtcaacacacaaggcgttcttccaggcatggtctggcaggacagagatgtgtaccttcaggggcccatctgggcaaagattccacacacggacggacattttcacccctctcccctcatgggtggattcggacttaaacaccctcctccacagattctcatcaagaacaccccggtacctgcgaatccttcgaccaccttcagtgcggcaaagtttgcttccttcatcacacagtactccacgggacaggtcagcgtggagatcgagtgggagctgcagaaggaaaacagcaaacgctggaatcccgaaattcagtacacttccaactacaacaagtctgttaatgtggactttactgtggacactaatggcgtgtattcagagcctcgccccattggcaccagatacctgactcgtaatctgtaa

SEQ ID NO: 29 - DNA, 2448 bp, Artificial Sequence
  Cap gene expression cassette
gacctttaattcaacccaacacaatatattatagttaaataagaattattatcaaatcatttgtatattaattaaaatactatactgtaaattacattttatttacaatcactcgacgaagacttgatcacccgggtcaggtagtaagtatcgataactttgttttctttcacatttacaactccgacatacaaatcccattacggcagtataaattcgttcattttggatattgtttcagtggctgccgacggttatctacccgattggctcgaggacactctctctgaaggaataagacagtggtggaagctcaaacctggcccaccaccaccaaagcccgcagagcggcataaggacgacagcaggggtcttgtgcttcctgggtacaagtacctcggacccttcaacggactcgacaagggagagccggtcaacgaggcagacgccgcggccctcgagcacgacaaagcctacgaccggcagctcgacagcggagacaacccgtacctcaagtacaaccacgccgacgcggagtttcaggagcgccttaaagaagatacgtcttttgggggcaacctcggacgagcagtcttccaggcgaaaaagagggttcttgaacctctgggcctggttgaggaacctgttaagacggctccgggaaaaaagaggccggtagagcactctcctgtggagccagactcctcctcgggaaccggaaaggcgggccagcagcctgcaagaaaaagattgaattttggtcagactggagacgcagactcagtacctgacccccagcctctcggacagccaccagcagccccctctggtctgggaactaatacgatggctacaggcagtggcgcaccaatggcagacaataacgagggcgccgacggagtgggtaattcctcgggaaattggcattgcgattccacatggatgggcgacagagtcatcaccaccagcacccgaacctgggccctgcccacctacaacaaccacctctacaaacaaatttccagccaatcaggagcctcgaacgacaatcactactttggctacagcaccccttgggggtattttgacttcaacagattccactgccacttttcaccacgtgactggcaaagactcatcaacaacaactggggattccgacccaagagactcaacttcaagctctttaacattcaagtcaaagaggtcacgcagaatgacggtacgacgacgattgccaataaccttaccagcacggttcaggtgtttactgactcggagtaccagctcccgtacgtcctcggctcggcgcatcaaggatgcctcccgccgttcccagcagacgtcttcatggtgccacagtatggatacctcaccctgaacaacgggagtcaggcagtaggacgctcttcattttactgcctggagtactttccttctcagatgctgcgtaccggaaacaactttaccttcagctacacttttgaggacgttcctttccacagcagctacgctcacagccagagtctggaccgtctcatgaatcctctcatcgaccagtacctgtattacttgagcagaacaaacactccaagtggaaccaccacgcagtcaaggcttcagttttctcaggccggagcgagtgacattcgggaccagtctaggaactggcttcctggaccctgttaccgccagcagcgagtatcaaagacatctgcggataacaacaacagtgaatactcgtggactggagctaccaagtaccacctcaatggcagagactctctggtgaatccgggcccggccatggcaagccacaaggacgatgaagaaaagttttttcctcagagcggggttctcatctttgggaagcaaggctcagagaaaacaaatgtggacattgaaaaggtcatgattacagacgaagaggaaatcaggacaaccaatcccgtggctacggagcagtatggttctgtatctaccaacctccagagaggcaacagacaagcagctaccgcagatgtcaacacacaaggcgttcttccaggcatggtctggcaggacagagatgtgtaccttcaggggcccatctgggcaaagattccacacacggacggacattttcacccctctcccctcatgggtggattcggacttaaacaccctcctccacagattctcatcaagaacaccccggtacctgcgaatccttcgaccaccttcagtgcggcaaagtttgcttccttcatcacacagtactccacgggacaggtcagcgtggagatcgagtgggagctgcagaaggaaaacagcaaacgctggaatcccgaaattcagtacacttccaactacaacaagtctgttaatgtggactttactgtggacactaatggcgtgtattcagagcctcgccccattggcaccagatacctgactcgtaatctgtaa

SEQ ID NO: 30 - DNA, 2569 bp, Artificial Sequence
  Cap gene expression cassette
gacctttaattcaacccaacacaatatattatagttaaataagaattattatcaaatcatttgtatattaattaaaatactatactgtaaattacattttatttacaatcactcgacgaagacttgatcacccgggtaggacaaggtaagtattcattgtaaatctgatattatttgtattattatacctacctaatttgcagtgcagataaatatgccggatggtaattttattactgtttggtccataaacacttgtttaccatttccttttttacaagttttaatatgttctgcatatataaaacattatgtattttgcagcaccttcaacggctcgggagaagggcggggaagcctcctaacctgcggtgacgttgaggaaaatccgggtccatcttttgttgatcacccacccgattggttggaagaagttggtgaaggtcttcgcgagtttttgggccttgaagcgggcccaccgaaaccaaaacccaatcagcagcatcaagatcaagcccgtggtcttgtgctgcctggttataactatctcggacccggaaacggtctcgatcgaggagagcctgtcaacagggcagacgaggtcgcgcgagagcacgacatctcgtacaacgagcagcttgaggcgggagacaacccctacctcaagtacaaccacgcggacgccgagtttcaggagaagctcgccgacgacacatccttcgggggaaacctcggaaaggcagtctttcaggccaagaaaagggttctcgaaccttttggcctggttgaagagggtgctaagacggcccctaccggaaagcggatagacgaccactttccaaaaagaaagaaggctcggaccgaagaggactccaagccttccacctcgtcagacgccgaagctggacccagcggatcccagcagctgcaaatcccagcccaaccagcctcaagtttgggagctgatacaatgtctgcgggaggtggcggcccattgggcgacaataaccaaggtgccgatggagtgggcaatgcctcgggagattggcattgcgattccacgtggatgggggacagagtcgtcaccaagtccacccgaacctgggtgctgcccagctacaacaaccaccagtaccgagagatcaaaagcggctccgtcgacggaagcaacgccaacgcctactttggatacagcaccccctgggggtactttgactttaaccgcttccacagccactggagcccccgagactggcaaagactcatcaacaactactggggcttcagaccccggtccctcagagtcaaaatcttcaacattcaagtcaaagaggtcacggtgcaggactccaccaccaccatcgccaacaacctcacctccaccgtccaagtgtttacggacgacgactaccagctgccctacgtcgtcggcaacgggaccgagggatgcctgccggccttccctccgcaggtctttacgctgccgcagtacggttacgcgacgctgaaccgcgacaacacagaaaatcccaccgagaggagcagcttcttctgcctagagtactttcccagcaagatgctgagaacgggcaacaactttgagtttacctacaactttgaggaggtgcccttccactccagcttcgctcccagtcagaacctcttcaagctggccaacccgctggtggaccagtacttgtaccgcttcgtgagcacaaataacactggcggagtccagttcaacaagaacctggccgggagatacgccaacacctacaaaaactggttcccggggcccatgggccgaacccagggctggaacctgggctccggggtcaaccgcgccagtgtcagcgccttcgccacgaccaataggatggagctcgagggcgcgagttaccaggtgcccccgcagccgaacggcatgaccaacaacctccagggcagcaacacctatgccctggagaacactatgatcttcaacagccagccggcgaacccgggcaccaccgccacgtacctcgagggcaacatgctcatcaccagcgagagcgagacgcagccggtgaaccgcgtggcgtacaacgtcggcgggcagatggccaccaacaaccagagctccaccactgcccccgcgaccggcacgtacaacctccaggaaatcgtgcccggcagcgtgtggatggagagggacgtgtacctccaaggacccatctgggccaagatcccagagacgggggcgcactttcacccctctccggccatgggcggattcggactcaaacacccaccgcccatgatgctcatcaagaacacgcctgtgcccggaaatatcaccagcttctcggacgtgcccgtcagcagcttcatcacccagtacagcaccgggcaggtcaccgtggagatggagtgggagctcaagaaggaaaactccaagaggtggaacccagagatccagtacacaaacaactacaacgacccccagtttgtggactttgccccggacagcaccggggaatacagaagcaccagacctatcggaacccgataccttacccgacccctttaa

SEQ ID NO: 31 - DNA, 2541 bp, Artificial Sequence
  Cap gene expression cassette
gacctttaattcaacccaacacaatatattatagttaaataagaattattatcaaatcatttgtatattaattaaaatactatactgtaaattacattttatttacaatcactcgacgaagacttgatcacccgggggacaaggtaagtattcattgtaaatctgatattatttgtattattatacctacctaatttgcagtgcaggccgccatggtaagtatcgataactttgttttctttcacatttacaactccgacatacaaattgtaattttattactgtttggtccataaacacttgtttaccatttccttttttacaagttttaatattttctgcatatataaaacattatttattttgcagtcttttgttgatcacccacccgattggttggaagaagttggtgaaggtcttcgcgagtttttgggccttgaagcgggcccaccgaaaccaaaacccaatcagcagcatcaagatcaagcccgtggtcttgtgctgcctggttataactatctcggacccggaaacggtctcgatcgaggagagcctgtcaacagggcagacgaggtcgcgcgagagcacgacatctcgtacaacgagcagcttgaggcgggagacaacccctacctcaagtacaaccacgcggacgccgagtttcaggagaagctcgccgacgacacatccttcgggggaaacctcggaaaggcagtctttcaggccaagaaaagggttctcgaaccttttggcctggttgaagagggtgctaagacggcccctaccggaaagcggatagacgaccactttccaaaaagaaagaaggctcggaccgaagaggactccaagccttccacctcgtcagacgccgaagctggacccagcggatcccagcagctgcaaatcccagcccaaccagcctcaagtttgggagctgatacaatgtctgcgggaggtggcggcccattgggcgacaataaccaaggtgccgatggagtgggcaatgcctcgggagattggcattgcgattccacgtggatgggggacagagtcgtcaccaagtccacccgaacctgggtgctgcccagctacaacaaccaccagtaccgagagatcaaaagcggctccgtcgacggaagcaacgccaacgcctactttggatacagcaccccctgggggtactttgactttaaccgcttccacagccactggagcccccgagactggcaaagactcatcaacaactactggggcttcagaccccggtccctcagagtcaaaatcttcaacattcaagtcaaagaggtcacggtgcaggactccaccaccaccatcgccaacaacctcacctccaccgtccaagtgtttacggacgacgactaccagctgccctacgtcgtcggcaacgggaccgagggatgcctgccggccttccctccgcaggtctttacgctgccgcagtacggttacgcgacgctgaaccgcgacaacacagaaaatcccaccgagaggagcagcttcttctgcctagagtactttcccagcaagatgctgagaacgggcaacaactttgagtttacctacaactttgaggaggtgcccttccactccagcttcgctcccagtcagaacctcttcaagctggccaacccgctggtggaccagtacttgtaccgcttcgtgagcacaaataacactggcggagtccagttcaacaagaacctggccgggagatacgccaacacctacaaaaactggttcccggggcccatgggccgaacccagggctggaacctgggctccggggtcaaccgcgccagtgtcagcgccttcgccacgaccaataggatggagctcgagggcgcgagttaccaggtgcccccgcagccgaacggcatgaccaacaacctccagggcagcaacacctatgccctggagaacactatgatcttcaacagccagccggcgaacccgggcaccaccgccacgtacctcgagggcaacatgctcatcaccagcgagagcgagacgcagccggtgaaccgcgtggcgtacaacgtcggcgggcagatggccaccaacaaccagagctccaccactgcccccgcgaccggcacgtacaacctccaggaaatcgtgcccggcagcgtgtggatggagagggacgtgtacctccaaggacccatctgggccaagatcccagagacgggggcgcactttcacccctctccggccatgggcggattcggactcaaacacccaccgcccatgatgctcatcaagaacacgcctgtgcccggaaatatcaccagcttctcggacgtgcccgtcagcagcttcatcacccagtacagcaccgggcaggtcaccgtggagatggagtgggagctcaagaaggaaaactccaagaggtggaacccagagatccagtacacaaacaactacaacgacccccagtttgtggactttgccccggacagcaccggggaatacagaagcaccagacctatcggaacccgataccttacccgacccctttaa

SEQ ID NO: 32 - DNA, 2415 bp, Artificial Sequence
  Cap gene expression cassette
gacctttaattcaacccaacacaatatattatagttaaataagaattattatcaaatcatttgtatattaattaaaatactatactgtaaattacattttatttacaatcactcgacgaagacttgatcacccgggtcaggtagtaagtatcgataactttgttttctttcacatttacaactccgacatacaaatcccattacggcagtataaattcgttcattttggatattgtttcagtgtcttttgttgatcacccacccgattggttggaagaagttggtgaaggtcttcgcgagtttttgggccttgaagcgggcccaccgaaaccaaaacccaatcagcagcatcaagatcaagcccgtggtcttgtgctgcctggttataactatctcggacccggaaacggtctcgatcgaggagagcctgtcaacagggcagacgaggtcgcgcgagagcacgacatctcgtacaacgagcagcttgaggcgggagacaacccctacctcaagtacaaccacgcggacgccgagtttcaggagaagctcgccgacgacacatccttcgggggaaacctcggaaaggcagtctttcaggccaagaaaagggttctcgaaccttttggcctggttgaagagggtgctaagacggcccctaccggaaagcggatagacgaccactttccaaaaagaaagaaggctcggaccgaagaggactccaagccttccacctcgtcagacgccgaagctggacccagcggatcccagcagctgcaaatcccagcccaaccagcctcaagtttgggagctgatacaatgtctgcgggaggtggcggcccattgggcgacaataaccaaggtgccgatggagtgggcaatgcctcgggagattggcattgcgattccacgtggatgggggacagagtcgtcaccaagtccacccgaacctgggtgctgcccagctacaacaaccaccagtaccgagagatcaaaagcggctccgtcgacggaagcaacgccaacgcctactttggatacagcaccccctgggggtactttgactttaaccgcttccacagccactggagcccccgagactggcaaagactcatcaacaactactggggcttcagaccccggtccctcagagtcaaaatcttcaacattcaagtcaaagaggtcacggtgcaggactccaccaccaccatcgccaacaacctcacctccaccgtccaagtgtttacggacgacgactaccagctgccctacgtcgtcggcaacgggaccgagggatgcctgccggccttccctccgcaggtctttacgctgccgcagtacggttacgcgacgctgaaccgcgacaacacagaaaatcccaccgagaggagcagcttcttctgcctagagtactttcccagcaagatgctgagaacgggcaacaactttgagtttacctacaactttgaggaggtgcccttccactccagcttcgctcccagtcagaacctcttcaagctggccaacccgctggtggaccagtacttgtaccgcttcgtgagcacaaataacactggcggagtccagttcaacaagaacctggccgggagatacgccaacacctacaaaaactggttcccggggcccatgggccgaacccagggctggaacctgggctccggggtcaaccgcgccagtgtcagcgccttcgccacgaccaataggatggagctcgagggcgcgagttaccaggtgcccccgcagccgaacggcatgaccaacaacctccagggcagcaacacctatgccctggagaacactatgatcttcaacagccagccggcgaacccgggcaccaccgccacgtacctcgagggcaacatgctcatcaccagcgagagcgagacgcagccggtgaaccgcgtggcgtacaacgtcggcgggcagatggccaccaacaaccagagctccaccactgcccccgcgaccggcacgtacaacctccaggaaatcgtgcccggcagcgtgtggatggagagggacgtgtacctccaaggacccatctgggccaagatcccagagacgggggcgcactttcacccctctccggccatgggcggattcggactcaaacacccaccgcccatgatgctcatcaagaacacgcctgtgcccggaaatatcaccagcttctcggacgtgcccgtcagcagcttcatcacccagtacagcaccgggcaggtcaccgtggagatggagtgggagctcaagaaggaaaactccaagaggtggaacccagagatccagtacacaaacaactacaacgacccccagtttgtggactttgccccggacagcaccggggaatacagaagcaccagacctatcggaacccgataccttacccgacccctttaa

SEQ ID NO: 33 - DNA, 2611 bp, Artificial Sequence
  Cap gene expression cassette
gacctttaattcaacccaacacaatatattatagttaaataagaattattatcaaatcatttgtatattaattaaaatactatactgtaaattacattttatttacaatcactcgacgaagacttgatcacccgggtaggacaaggtaagtattcattgtaaatctgatattatttgtattattatacctacctaatttgcagtgcagataaatatgccggatggtaattttattactgtttggtccataaacacttgtttaccatttccttttttacaagttttaatatgttctgcatatataaaacattatgtattttgcagcaccttcaacggctcgggagaagggcggggaagcctcctaacctgcggtgacgttgaggaaaatccgggtccagctgccgacggttatctacccgattggctcgaggacaacctctctgagggcattcgcgagtggtgggcgctgaaacctggagccccgaagcccaaagccaaccagcaaaagcaggacgacggccggggtctggtgcttcctggctacaagtacctcggacccttcaacggactcgacaagggggagcccgtcaacgcggcggacgcagcggccctcgagcacgacaaggcctacgaccagcagctgcaggcgggtgacaatccgtacctgcggtataaccacgccgacgccgagtttcaggagcgtctgcaagaagatacgtcttttgggggcaacctcgggcgagcagtcttccaggccaagaagcgggttctcgaacctctcggtctggttgaggaaggcgctaagacggctcctggaaagaagagaccggtagagccatcaccccagcgttctccagactcctctacgggcatcggcaagaaaggccaacagcccgccagaaaaagactcaattttggtcagactggcgactcagagtcagttccagaccctcaacctctcggagaacctccagcagcgccctctggtgtgggacctaatacaatggctgcaggcggtggcgcaccaatggcagacaataacgaaggcgccgacggagtgggtagttcctcgggaaattggcattgcgattccacatggctgggcgacagagtcatcaccaccagcacccgaacctgggccctgcccacctacaacaaccacctctacaagcaaatctccaacgggacatcgggaggagccaccaacgacaacacctacttcggctacagcaccccctgggggtattttgactttaacagattccactgccacttttcaccacgtgactggcagcgactcatcaacaacaactggggattccggcccaagagactcagcttcaagctcttcaacatccaggtcaaggaggtcacgcagaatgaaggcaccaagaccatcgccaataacctcaccagcaccatccaggtgtttacggactcggagtaccagctgccgtacgttctcggctctgcccaccagggctgcctgcctccgttcccggcggacgtgttcatgattccccagtacggctacctaacactcaacaacggtagtcaggccgtgggacgctcctccttctactgcctggaatactttccttcgcagatgctgagaaccggcaacaacttccagtttacttacaccttcgaggacgtgcctttccacagcagctacgcccacagccagagcttggaccggctgatgaatcctctgattgaccagtacctgtactacttgtctcggactcaaacaacaggaggcacggcaaatacgcagactctgggcttcagccaaggtgggcctaatacaatggccaatcaggcaaagaactggctgccaggaccctgttaccgccaacaacgcgtctcaacgacaaccgggcaaaacaacaatagcaactttgcctggactgctgggaccaaataccatctgaatggaagaaattcattggctaatcctggcatcgctatggcaacacacaaagacgacgaggagcgtttttttcccagtaacgggatcctgatttttggcaaacaaaatgctgccagagacaatgcggattacagcgatgtcatgctcaccagcgaggaagaaatcaaaaccactaaccctgtggctacagaggaatacggtatcgtggcagataacttgcagcagcaaaacacggctcctcaaattggaactgtcaacagccagggggccttacccggtatggtctggcagaaccgggacgtgtacctgcagggtcccatctgggccaagattcctcacacggacggcaacttccacccgtctccgctgatgggcggctttggcctgaaacatcctccgcctcagatcctgatcaagaacacgcctgtacctgcggatcctccgaccaccttcaaccagtcaaagctgaactctttcatcacgcaatacagcaccggacaggtcagcgtggaaattgaatgggagctgcagaaggaaaacagcaagcgctggaaccccgagatccagtacacctccaactactacaaatctacaagtgtggactttgctgttaatacagaaggcgtgtactctgaaccccgccccattggcacccgttacctcacccgtaatctgtaa

SEQ ID NO: 34 - DNA, 2583 bp, Artificial Sequence
  Cap gene expression cassette
gacctttaattcaacccaacacaatatattatagttaaataagaattattatcaaatcatttgtatattaattaaaatactatactgtaaattacattttatttacaatcactcgacgaagacttgatcacccgggggacaaggtaagtattcattgtaaatctgatattatttgtattattatacctacctaatttgcagtgcaggccgccatggtaagtatcgataactttgttttctttcacatttacaactccgacatacaaattgtaattttattactgtttggtccataaacacttgtttaccatttccttttttacaagttttaatattttctgcatatataaaacattatttattttgcaggctgccgacggttatctacccgattggctcgaggacaacctctctgagggcattcgcgagtggtgggcgctgaaacctggagccccgaagcccaaagccaaccagcaaaagcaggacgacggccggggtctggtgcttcctggctacaagtacctcggacccttcaacggactcgacaagggggagcccgtcaacgcggcggacgcagcggccctcgagcacgacaaggcctacgaccagcagctgcaggcgggtgacaatccgtacctgcggtataaccacgccgacgccgagtttcaggagcgtctgcaagaagatacgtcttttgggggcaacctcgggcgagcagtcttccaggccaagaagcgggttctcgaacctctcggtctggttgaggaaggcgctaagacggctcctggaaagaagagaccggtagagccatcaccccagcgttctccagactcctctacgggcatcggcaagaaaggccaacagcccgccagaaaaagactcaattttggtcagactggcgactcagagtcagttccagaccctcaacctctcggagaacctccagcagcgccctctggtgtgggacctaatacaatggctgcaggcggtggcgcaccaatggcagacaataacgaaggcgccgacggagtgggtagttcctcgggaaattggcattgcgattccacatggctgggcgacagagtcatcaccaccagcacccgaacctgggccctgcccacctacaacaaccacctctacaagcaaatctccaacgggacatcgggaggagccaccaacgacaacacctacttcggctacagcaccccctgggggtattttgactttaacagattccactgccacttttcaccacgtgactggcagcgactcatcaacaacaactggggattccggcccaagagactcagcttcaagctcttcaacatccaggtcaaggaggtcacgcagaatgaaggcaccaagaccatcgccaataacctcaccagcaccatccaggtgtttacggactcggagtaccagctgccgtacgttctcggctctgcccaccagggctgcctgcctccgttcccggcggacgtgttcatgattccccagtacggctacctaacactcaacaacggtagtcaggccgtgggacgctcctccttctactgcctggaatactttccttcgcagatgctgagaaccggcaacaacttccagtttacttacaccttcgaggacgtgcctttccacagcagctacgcccacagccagagcttggaccggctgatgaatcctctgattgaccagtacctgtactacttgtctcggactcaaacaacaggaggcacggcaaatacgcagactctgggcttcagccaaggtgggcctaatacaatggccaatcaggcaaagaactggctgccaggaccctgttaccgccaacaacgcgtctcaacgacaaccgggcaaaacaacaatagcaactttgcctggactgctgggaccaaataccatctgaatggaagaaattcattggctaatcctggcatcgctatggcaacacacaaagacgacgaggagcgtttttttcccagtaacgggatcctgatttttggcaaacaaaatgctgccagagacaatgcggattacagcgatgtcatgctcaccagcgaggaagaaatcaaaaccactaaccctgtggctacagaggaatacggtatcgtggcagataacttgcagcagcaaaacacggctcctcaaattggaactgtcaacagccagggggccttacccggtatggtctggcagaaccgggacgtgtacctgcagggtcccatctgggccaagattcctcacacggacggcaacttccacccgtctccgctgatgggcggctttggcctgaaacatcctccgcctcagatcctgatcaagaacacgcctgtacctgcggatcctccgaccaccttcaaccagtcaaagctgaactctttcatcacgcaatacagcaccggacaggtcagcgtggaaattgaatgggagctgcagaaggaaaacagcaagcgctggaaccccgagatccagtacacctccaactactacaaatctacaagtgtggactttgctgttaatacagaaggcgtgtactctgaaccccgccccattggcacccgttacctcacccgtaatctgtaa

SEQ ID NO: 35 - DNA, 2457 bp, Artificial Sequence
  Cap gene expression cassette
gacctttaattcaacccaacacaatatattatagttaaataagaattattatcaaatcatttgtatattaattaaaatactatactgtaaattacattttatttacaatcactcgacgaagacttgatcacccgggtcaggtagtaagtatcgataactttgttttctttcacatttacaactccgacatacaaatcccattacggcagtataaattcgttcattttggatattgtttcagtggctgccgacggttatctacccgattggctcgaggacaacctctctgagggcattcgcgagtggtgggcgctgaaacctggagccccgaagcccaaagccaaccagcaaaagcaggacgacggccggggtctggtgcttcctggctacaagtacctcggacccttcaacggactcgacaagggggagcccgtcaacgcggcggacgcagcggccctcgagcacgacaaggcctacgaccagcagctgcaggcgggtgacaatccgtacctgcggtataaccacgccgacgccgagtttcaggagcgtctgcaagaagatacgtcttttgggggcaacctcgggcgagcagtcttccaggccaagaagcgggttctcgaacctctcggtctggttgaggaaggcgctaagacggctcctggaaagaagagaccggtagagccatcaccccagcgttctccagactcctctacgggcatcggcaagaaaggccaacagcccgccagaaaaagactcaattttggtcagactggcgactcagagtcagttccagaccctcaacctctcggagaacctccagcagcgccctctggtgtgggacctaatacaatggctgcaggcggtggcgcaccaatggcagacaataacgaaggcgccgacggagtgggtagttcctcgggaaattggcattgcgattccacatggctgggcgacagagtcatcaccaccagcacccgaacctgggccctgcccacctacaacaaccacctctacaagcaaatctccaacgggacatcgggaggagccaccaacgacaacacctacttcggctacagcaccccctgggggtattttgactttaacagattccactgccacttttcaccacgtgactggcagcgactcatcaacaacaactggggattccggcccaagagactcagcttcaagctcttcaacatccaggtcaaggaggtcacgcagaatgaaggcaccaagaccatcgccaataacctcaccagcaccatccaggtgtttacggactcggagtaccagctgccgtacgttctcggctctgcccaccagggctgcctgcctccgttcccggcggacgtgttcatgattccccagtacggctacctaacactcaacaacggtagtcaggccgtgggacgctcctccttctactgcctggaatactttccttcgcagatgctgagaaccggcaacaacttccagtttacttacaccttcgaggacgtgcctttccacagcagctacgcccacagccagagcttggaccggctgatgaatcctctgattgaccagtacctgtactacttgtctcggactcaaacaacaggaggcacggcaaatacgcagactctgggcttcagccaaggtgggcctaatacaatggccaatcaggcaaagaactggctgccaggaccctgttaccgccaacaacgcgtctcaacgacaaccgggcaaaacaacaatagcaactttgcctggactgctgggaccaaataccatctgaatggaagaaattcattggctaatcctggcatcgctatggcaacacacaaagacgacgaggagcgtttttttcccagtaacgggatcctgatttttggcaaacaaaatgctgccagagacaatgcggattacagcgatgtcatgctcaccagcgaggaagaaatcaaaaccactaaccctgtggctacagaggaatacggtatcgtggcagataacttgcagcagcaaaacacggctcctcaaattggaactgtcaacagccagggggccttacccggtatggtctggcagaaccgggacgtgtacctgcagggtcccatctgggccaagattcctcacacggacggcaacttccacccgtctccgctgatgggcggctttggcctgaaacatcctccgcctcagatcctgatcaagaacacgcctgtacctgcggatcctccgaccaccttcaaccagtcaaagctgaactctttcatcacgcaatacagcaccggacaggtcagcgtggaaattgaatgggagctgcagaaggaaaacagcaagcgctggaaccccgagatccagtacacctccaactactacaaatctacaagtgtggactttgctgttaatacagaaggcgtgtactctgaaccccgccccattggcacccgttacctcacccgtaatctgtaa

SEQ ID NO: 36 - protein, 18 aa, Thosea asigna virus
  Self-cleaving peptides T2A
EGRGSLLTCGDVEENPGP

SEQ ID NO: 37 - protein, 19 aa, Porcine teschovirus
  Self-cleaving peptides P2A
ATNFSLLKQAGDVEENPGP

SEQ ID NO: 38 - protein, 20 aa, Equine rhinitis A virus
  Self-cleaving peptides E2A
QCTNYALLKLAGDVESNPGP

SEQ ID NO: 39 - protein, 22 aa, Foot-and-mouth disease virus
  Self-cleaving peptides F2A
VKQTLNFDLLKLAGDVESNPGP